European Patent Application EP 4 349 975 A1, published April 10, 2024. Title: CHIMERIC BROAD-SPECTRUM ONCOLYTIC ADENOVIRUS WITH MULTIPLE MECHANISMS SYNERGIZING WITH AND ENHANCING EFFICACY OF IMMUNOTHERAPY, AND APPLICATION THEREOF IN TUMOR TREATMENT. Applicant: VONCOLYTIC THERAPEUTICS CO., LTD. The sequence listing filed with the application follows.

SEQUENCE LISTING (3 sequences)

SEQ ID NO: 1 - DNA, 949 bp, Artificial Sequence
  sequence of attR1+ccdB+attR2
taaacaagtttgtacaaaaaagctgaacgagaaacgtaaaatgatataaatatcaatatattaaattagattttgcataaaaaacagactacataatactgtaaaacacaacatatccagtcactatggcggccgatctggatccggcttactaaaagccagataacagtatgcgtatttgcgcgctgatttttgcggtataagaatatatactgatatgtatacccgaagtatgtcaaaaagaggtgtgctatgaagcagcgtattacagtgacagttgacagcgacagctatcagttgctcaaggcatatatgatgtcaatatctccggtctggtaagcacaaccatgcagaatgaagcccgtcgtctgcgtgccgaacgctggaaagcggaaaatcaggaagggatggctgaggtcgcccggtttattgaaatgaacggctcttttgctgacgagaacagggactggtgaaatgcagtttaaggtttacacctataaaagagagagccgttatcgtctgtttgtggatgtacagagtgatattattgacacgcccgggcgacggatggtgatccccctggccagtgcacgtctgctgtcagataaagtctcccgtgaactttacccggtggtgcatatcggggatgaaagctggcgcatgatgaccaccgatatggccagtgtgccggtctccgttatcggggaagaagtggctgatctcagccaccgcgaaaatgacatcaaaaacgccattaacctgatgttctggggaatataaatgtcaggctcccttatacacagccagtctgcaggtcgaccatagtgactggatatgttgtgttttacagtattatgtagtctgttttttatgcaaaatctaatttaatatattgatatttatatcattttacgtttctcgttcagctttcttgtacaaagtggttaat

SEQ ID NO: 2 - DNA, 769 bp, Artificial Sequence
  mCMV promoter+SpeI/EcoRI/HindIII/BglII/NheI/BamHI/SalI+Poly(A)
ccatggctctagagatatactgagtcattagggactttccaatgggttttgcccagtacataaggtcaataggggtgaatcaacaggaaagtcccattggagccaagtacactgagtcaatagggactttccattgggttttgcccagtacaaaaggtcaatagggggtgagtcaatgggtttttcccattattggcacgtacataaggtcaataggggtgagtcattgggtttttccagccatttaattaaaacgccatgtactttcccaccattgacgtcaatgggctattgaaactaatgcaacgtgacctttaaacggtactttcccatagctgattaatgggaaagtaccgttctcgagccaatacacgtcaatgggaagtgaaagggcagccaaaacgtaacaccgccccggttttcccctggaaattccatattggcactcattctattggctgagctgcgttctacgtgggtataagaggcgcgaccagcgtcggtaccgtcgcagtcttcggtctgaccaccgtagaacgcagatcgaattactagtcagggaattcaagcttagatctgctagcaaggatccagcttgtcgacttcgagcaacttgtttattgcagcttataatggttacaaataaagcaatagcatcacaaatttcacaaataaagcatttttttcactgcattctagttgtggtttgtccaaactcatcaatgtatcttatcatgtctggatcgtctagcatcgaagatccgatatc

SEQ ID NO: 3 - DNA, 37515 bp, Artificial Sequence
  full genome sequence of VirRon
ttattttggattgaagccaatatgataatgagggggtggagtttgtgacgtggcgcggggcgtgggaacggggcgggtgacgtagtagtgtggcggaagtgtgatgttgcaagtgtggcggaacacatgtaagcgacggatgtggcaaaagtgacgtttttggtgtgcgccggtgtacacaggaagtgacaattttcgcgcggttttaggcggatgttgtagtaaatttgggcgtaaccgagtaagatttggccattttcgcgggaaaactgaataagaggaagtgaaatctgaataattttgtgttactcatagcgcgtaatatttgtctagggccgcggggactttgaccgtttacgtggagactcgcccaggtgtttttctcaggtgttttccgcgttccgggtcaaagttggcgttttattattatagtcagctgacgtgtaaccggcgtacgttcggccgcagatctggtcgactagtccatataaggtataaatccatataaggtataaatccatataaggtaataggctgcaggacttactgttggtgggacgccctgctttgcgaagggaaaggaggagtttgccctgagcacaggcccccaccctccactgggctttccccagctcccttgtcttcttatcacggtagtggcccagtccctggcccctgactccagaaggtggccctcctggaaacccaggtcgtgcagtcaacgatgtactcgccgggacagcgatgtctgctgcactccatccctcccctgttcatttgtccttcatgcccgtctggagtagatgctttttgcagaggtggcaccctgtaaagctctcctgtctgactttttttttttttttagactgagttttgctcttgttgcctaggctggagtgcaatggcacaatctcagctcactgcaccctctgcctcccgggttcaagcgattctcctgcctcagcctcccgagtagttgggattacaggcatgcaccaccacgcccagctaatttttgtatttttagtagagacaaggtttcaccgtgatggccaggctggtcttgaactccaggactcaagtgatgctcctgcctaggcctctcaaagtgttgggattacaggcgtgagccactgcacccggcctgcacgcgttctttgaaagcagtcgagggggcgctaggtgtgggcagggacgagctggcgcggcgtcgctgggtgcaccgcgaccacgggcagagccacgcggcgggaggactacaactcccggcacaccccgcgccgccccgcctctactcccagaaggccgcggggggtggaccgcctaagagggcgtgcgctcccgacatgccccgcggcgcgccattaaccgccagatttgaatcgcgggacaccgggactgaaaatgagacatattatctgccacggaggtgttattaccgaagaaatggccgccagtcttttggaccagctgatcgaagaggtactggctgataatcttccacctcctagccattttgaaccacctacccttcacgaactgtatgatttagacgtgacggcccccgaagatcccaacgaggaggcggtttcgcagatttttcccgactctgtaatgttggcggtgcaggaagggattgacttactcacttttccgccggcgcccggttctccggagccgcctcacctttcccggcagcccgagcagccggagcagagagccttgggtccggtttctatgccaaaccttgtaccggaggtgatcgatcttacctgctttccacccagtgacgacgaggatgaagagggtgaggagtttgtgttagattatgtggagcaccccgggcacggttgcaggtcttgtcattatcaccggaggaatacgggggacccagatattatgtgttcgctttgctatatgaggacctgtggcatgtttgtctacagtaagtgaaaattatgggcagtgggtgatagagtggtgggtttggtgtggtaattttttttttaatttttacagttttgtggtttaaagaattttgtattgtgatttttttaaaaggtcctgtgtctgaacctgagcctgagcccgagccagaaccggagcctgcaagacctacccgccgtcctaaaatggcgcctgctatcctgagacgcccgacatcacctgtgtctagagaatgcaatagtagtacggatagctgtgactccggtccttctaacacacctcctgagatacacccggtggtcccgctgtgccccattaaaccagttgccgtgagagttggtgggcgtcgccaggctgtggaatgtatcgaggacttgcttaacgagcctgggcaacctttggacttgagctgtaaacgccccaggccagacttggagatgttagctccctatatcccaatggatgatgacttccagtaacttgcatggcgtgttaaatggggcggggcttaaagggtatataatgcgccgtgggctaatcttggttacatctgacctcccggcgggtccggcgggtcaccatggagctcctcgactgataagcagatttgcacattagcattaacagatgtagctaagcactttgcttcagttctcatcagcactttatagtgacttccagatgtagctaagcactttgcttcagttctcaattagcattaatcagcactttctagtgacttcgagctcctcgactgataagcagatttgcactcagcactttgtagtgacttccagatgtagctaagcactttggagctcctcgactgataagcagatttgcaccttcagttctcaattagcattaaagatctggaaggtgctgaggtacgatgagacccgcaccaggtgcagaccctgcgagtgtggcggtaaacatattaggaaccagcctgtgatgctggatgtgaccgaggagctgaggcccgatcacttggtgctggcctgcacccgcgctgagtttggctctagcgatgaagatacagattgaggtactgaaatgtgtgggcgtggcttaagggtgggaaagaatatataaggtgggggtcttatgtagttttgtatctgttttgcagcagccgccgccgccatgagcaccaactcgtttgatggaagcattgtgagctcatatttgacaacgcgcatgcccccatgggccggggtgcgtcagaatgtgatgggctccagcattgatggtcgccccgtcctgcccgcaaactctactaccttgacctacgagaccgtgtctggaacgccgttggagactgcagcctccgccgccgcttcagccgctgcagccaccgcccgcgggattgtgactgactttgctttcctgagcccgcttgcaagcagtgcagcttcccgttcatccgcccgcgatgacaagttgacggctcttttggcacaattggattctttgacccgggaacttaatgtcgtttctcagcagctgttggatctgcgccagcaggtttctgccctgaaggcttcctcccctcccaatgcggtttaaaacataaataaaaaaccagactctgtttggatttggatcaagcaagtgtcttgctgtctttatttaggggttttgcgcgcgcggtaggcccgggaccagcggtctcggtcgttgagggtcctgtgtattttttccaggacgtggtaaaggtgactctggatgttcagatacatgggcataagcccgtctctggggtggaggtagcaccactgcagagcttcatgctgcggggtggtgttgtagatgatccagtcgtagcaggagcgctgggcgtggtgcctaaaaatgtctttcagtagcaagctgattgccaggggcaggcccttggtgtaagtgtttacaaagcggttaagctgggatgggtgcatacgtggggatatgagatgcatcttggactgtatttttaggttggctatgttcccagccatatccctccggggattcatgttgtgcagaaccaccagcacagtgtatccggtgcacttgggaaatttgtcatgtagcttagaaggaaatgcgtggaagaacttggagacgcccttgtgacctccaagattttccatgcattcgtccataatgatggcaatgggcccacgggcggcggcctgggcgaagatatttctgggatcactaacgtcatagttgtgttccaggatgagatcgtcataggccatttttacaaagcgcgggcggagggtgccagactgcggtataatggttccatccggcccaggggcgtagttaccctcacagatttgcatttcccacgctttgagttcagatggggggatcatgtctacctgcggggcgatgaagaaaacggtttccggggtaggggagatcagctgggaagaaagcaggttcctgagcagctgcgacttaccgcagccggtgggcccgtaaatcacacctattaccgggtgcaactggtagttaagagagctgcagctgccgtcatccctgagcaggggggccacttcgttaagcatgtccctgactcgcatgttttccctgaccaaatccgccagaaggcgctcgccgcccagcgatagcagttcttgcaaggaagcaaagtttttcaacggtttgagaccgtccgccgtaggcatgcttttgagcgtttgaccaagcagttccaggcggtcccacagctcggtcacctgctctacggcatctcgatccagcatatctcctcgtttcgcgggttggggcggctttcgctgtacggcagtagtcggtgctcgtccagacgggccagggtcatgtctttccacgggcgcagggtcctcgtcagcgtagtctgggtcacggtgaaggggtgcgctccgggctgcgcgctggccagggtgcgcttgaggctggtcctgctggtgctgaagcgctgccggtcttcgccctgcgcgtcggccaggtagcatttgaccatggtgtcatagtccagcccctccgcggcgtggcccttggcgcgcagcttgcccttggaggaggcgccgcacgaggggcagtgcagacttttgagggcgtagagcttgggcgcgagaaataccgattccggggagtaggcatccgcgccgcaggccccgcagacggtctcgcattccacgagccaggtgagctctggccgttcggggtcaaaaaccaggtttcccccatgctttttgatgcgtttcttacctctggtttccatgagccggtgtccacgctcggtgacgaaaaggctgtccgtgtccccgtatacagacttgagaggcctgtcctcgagcggtgttccgcggtcctcctcgtatagaaactcggaccactctgagacaaaggctcgcgtccaggccagcacgaaggaggctaagtgggaggggtagcggtcgttgtccactagggggtccactcgctccagggtgtgaagacacatgtcgccctcttcggcatcaaggaaggtgattggtttgtaggtgtaggccacgtgaccgggtgttcctgaaggggggctataaaagggggtgggggcgcgttcgtcctcactctcttccgcatcgctgtctgcgagggccagctgttggggtgagtactccctctgaaaagcgggcatgacttctgcgctaagattgtcagtttccaaaaacgaggaggatttgatattcacctggcccgcggtgatgcctttgagggtggccgcatccatctggtcagaaaagacaatctttttgttgtcaagcttggtggcaaacgacccgtagagggcgttggacagcaacttggcgatggagcgcagggtttggtttttgtcgcgatcggcgcgctccttggccgcgatgtttagctgcacgtattcgcgcgcaacgcaccgccattcgggaaagacggtggtgcgctcgtcgggcaccaggtgcacgcgccaaccgcggttgtgcagggtgacaaggtcaacgctggtggctacctctccgcgtaggcgctcgttggtccagcagaggcggccgcccttgcgcgagcagaatggcggtagggggtctagctgcgtctcgtccggggggtctgcgtccacggtaaagaccccgggcagcaggcgcgcgtcgaagtagtctatcttgcatccttgcaagtctagcgcctgctgccatgcgcgggcggcaagcgcgcgctcgtatgggttgagtgggggaccccatggcatggggtgggtgagcgcggaggcgtacatgccgcaaatgtcgtaaacgtagaggggctctctgagtattccaagatatgtagggtagcatcttccaccgcggatgctggcgcgcacgtaatcgtatagttcgtgcgagggagcgaggaggtcgggaccgaggttgctacgggcgggctgctctgctcggaagactatctgcctgaagatggcatgtgagttggatgatatggttggacgctggaagacgttgaagctggcgtctgtgagacctaccgcgtcacgcacgaaggaggcgtaggagtcgcgcagcttgttgaccagctcggcggtgacctgcacgtctagggcgcagtagtccagggtttccttgatgatgtcatacttatcctgtcccttttttttccacagctcgcggttgaggacaaactcttcgcggtctttccagtactcttggatcggaaacccgtcggcctccgaacggtaagagcctagcatgtagaactggttgacggcctggtaggcgcagcatcccttttctacgggtagcgcgtatgcctgcgcggccttccggagcgaggtgtgggtgagcgcaaaggtgtccctgaccatgactttgaggtactggtatttgaagtcagtgtcgtcgcatccgccctgctcccagagcaaaaagtccgtgcgctttttggaacgcggatttggcagggcgaaggtgacatcgttgaagagtatctttcccgcgcgaggcataaagttgcgtgtgatgcggaagggtcccggcacctcggaacggttgttaattacctgggcggcgagcacgatctcgtcaaagccgttgatgttgtggcccacaatgtaaagttccaagaagcgcgggatgcccttgatggaaggcaattttttaagttcctcgtaggtgagctcttcaggggagctgagcccgtgctctgaaagggcccagtctgcaagatgagggttggaagcgacgaatgagctccacaggtcacgggccattagcatttgcaggtggtcgcgaaaggtcctaaactggcgacctatggccattttttctggggtgatgcagtagaaggtaagcgggtcttgttcccagcggtcccatccaaggttcgcggctaggtctcgcgcggcagtcactagaggctcatctccgccgaacttcatgaccagcatgaagggcacgagctgcttcccaaaggcccccatccaagtataggtctctacatcgtaggtgacaaagagacgctcggtgcgaggatgcgagccgatcgggaagaactggatctcccgccaccaattggaggagtggctattgatgtggtgaaagtagaagtccctgcgacgggccgaacactcgtgctggcttttgtaaaaacgtgcgcagtactggcagcggtgcacgggctgtacatcctgcacgaggttgacctgacgaccgcgcacaaggaagcagagtgggaatttgagcccctcgcctggcgggtttggctggtggtcttctacttcggctgcttgtccttgaccgtctggctgctcgaggggagttacggtggatcggaccaccacgccgcgcgagcccaaagtccagatgtccgcgcgcggcggtcggagcttgatgacaacatcgcgcagatgggagctgtccatggtctggagctcccgcggcgtcaggtcaggcgggagctcctgcaggtttacctcgcatagacgggtcagggcgcgggctagatccaggtgatacctaatttccaggggctggttggtggcggcgtcgatggcttgcaagaggccgcatccccgcggcgcgactacggtaccgcgcggcgggcggtgggccgcgggggtgtccttggatgatgcatctaaaagcggtgacgcgggcgagcccccggaggtagggggggctccggacccgccgggagagggggcaggggcacgtcggcgccgcgcgcgggcaggagctggtgctgcgcgcgtaggttgctggcgaacgcgacgacgcggcggttgatctcctgaatctggcgcctctgcgtgaagacgacgggcccggtgagcttgagcctgaaagagagttcgacagaatcaatttcggtgtcgttgacggcggcctggcgcaaaatctcctgcacgtctcctgagttgtcttgataggcgatctcggccatgaactgctcgatctcttcctcctggagatctccgcgtccggctcgctccacggtggcggcgaggtcgttggaaatgcgggccatgagctgcgagaaggcgttgaggcctccctcgttccagacgcggctgtagaccacgcccccttcggcatcgcgggcgcgcatgaccacctgcgcgagattgagctccacgtgccgggcgaagacggcgtagtttcgcaggcgctgaaagaggtagttgagggtggtggcggtgtgttctgccacgaagaagtacataacccagcgtcgcaacgtggattcgttgatatcccccaaggcctcaaggcgctccatggcctcgtagaagtccacggcgaagttgaaaaactgggagttgcgcgccgacacggttaactcctcctccagaagacggatgagctcggcgacagtgtcgcgcacctcgcgctcaaaggctacaggggcctcttcttcttcttcaatctcctcttccataagggcctccccttcttcttcttctggcggcggtgggggaggggggacacggcggcgacgacggcgcaccgggaggcggtcgacaaagcgctcgatcatctccccgcggcgacggcgcatggtctcggtgacggcgcggccgttctcgcgggggcgcagttggaagacgccgcccgtcatgtcccggttatgggttggcggggggctgccatgcggcagggatacggcgctaacgatgcatctcaacaattgttgtgtaggtactccgccgccgagggacctgagcgagtccgcatcgaccggatcggaaaacctctcgagaaaggcgtctaaccagtcacagtcgcaaggtaggctgagcaccgtggcgggcggcagcgggcggcggtcggggttgtttctggcggaggtgctgctgatgatgtaattaaagtaggcggtcttgagacggcggatggtcgacagaagcaccatgtccttgggtccggcctgctgaatgcgcaggcggtcggccatgccccaggcttcgttttgacatcggcgcaggtctttgtagtagtcttgcatgagcctttctaccggcacttcttcttctccttcctcttgtcctgcatctcttgcatctatcgctgcggcggcggcggagtttggccgtaggtggcgccctcttcctcccatgcgtgtgaccccgaagcccctcatcggctgaagcagggctaggtcggcgacaacgcgctcggctaatatggcctgctgcacctgcgtgagggtagactggaagtcatccatgtccacaaagcggtggtatgcgcccgtgttgatggtgtaagtgcagttggccataacggaccagttaacggtctggtgacccggctgcgagagctcggtgtacctgagacgcgagtaagccctcgagtcaaatacgtagtcgttgcaagtccgcaccaggtactggtatcccaccaaaaagtgcggcggcggctggcggtagaggggccagcgtagggtggccggggctccgggggcgagatcttccaacataaggcgatgatatccgtagatgtacctggacatccaggtgatgccggcggcggtggtggaggcgcgcggaaagtcgcggacgcggttccagatgttgcgcagcggcaaaaagtgctccatggtcgggacgctctggccggtcaggcgcgcgcaatcgttgacgctctaccgtgcaaaaggagagcctgtaagcgggcactcttccgtggtctggtggataaattcgcaagggtatcatggcggacgaccggggttcgagccccgtatccggccgtccgccgtgatccatgcggttaccgcccgcgtgtcgaacccaggtgtgcgacgtcagacaacgggggagtgctccttttggcttccttccaggcgcggcggctgctgcgctagcttttttggccactggccgcgcgcagcgtaagcggttaggctggaaagcgaaagcattaagtggctcgctccctgtagccggagggttattttccaagggttgagtcgcgggacccccggttcgagtctcggaccggccggactgcggcgaacgggggtttgcctccccgtcatgcaagaccccgcttgcaaattcctccggaaacagggacgagccccttttttgcttttcccagatgcatccggtgctgcggcagatgcgcccccctcctcagcagcggcaagagcaagagcagcggcagacatgcagggcaccctcccctcctcctaccgcgtcaggaggggcgacatccgcggttgacgcggcagcagatggtgattacgaacccccgcggcgccgggcccggcactacctggacttggaggagggcgagggcctggcgcggctaggagcgccctctcctgagcggtacccaagggtgcagctgaagcgtgatacgcgtgaggcgtacgtgccgcggcagaacctgtttcgcgaccgcgagggagaggagcccgaggagatgcgggatcgaaagttccacgcagggcgcgagctgcggcatggcctgaatcgcgagcggttgctgcgcgaggaggactttgagcccgacgcgcgaaccgggattagtcccgcgcgcgcacacgtggcggccgccgacctggtaaccgcatacgagcagacggtgaaccaggagattaactttcaaaaaagctttaacaaccacgtgcgtacgcttgtggcgcgcgaggaggtggctataggactgatgcatctgtgggactttgtaagcgcgctggagcaaaacccaaatagcaagccgctcatggcgcagctgttccttatagtgcagcacagcagggacaacgaggcattcagggatgcgctgctaaacatagtagagcccgagggccgctggctgctcgatttgataaacatcctgcagagcatagtggtgcaggagcgcagcttgagcctggctgacaaggtggccgccatcaactattccatgcttagcctgggcaagttttacgcccgcaagatataccataccccttacgttcccatagacaaggaggtaaagatcgaggggttctacatgcgcatggcgctgaaggtgcttaccttgagcgacgacctgggcgtttatcgcaacgagcgcatccacaaggccgtgagcgtgagccggcggcgcgagctcagcgaccgcgagctgatgcacagcctgcaaagggccctggctggcacgggcagcggcgatagagaggccgagtcctactttgacgcgggcgctgacctgcgctgggccccaagccgacgcgccctggaggcagctggggccggacctgggctggcggtggcacccgcgcgcgctggcaacgtcggcggcgtggaggaatatgacgaggacgatgagtacgagccagaggacggcgagtactaagcggtgatgtttctgatcagatgatgcaagacgcaacggacccggcggtgcgggcggcgctgcagagccagccgtccggccttaactccacggacgactggcgccaggtcatggaccgcatcatgtcgctgactgcgcgcaatcctgacgcgttccggcagcagccgcaggccaaccggctctccgcaattctggaagcggtggtcccggcgcgcgcaaaccccacgcacgagaaggtgctggcgatcgtaaacgcgctggccgaaaacagggccatccggcccgacgaggccggcctggtctacgacgcgctgcttcagcgcgtggctcgttacaacagcggcaacgtgcagaccaacctggaccggctggtgggggatgtgcgcgaggccgtggcgcagcgtgagcgcgcgcagcagcagggcaacctgggctccatggttgcactaaacgccttcctgagtacacagcccgccaacgtgccgcggggacaggaggactacaccaactttgtgagcgcactgcggctaatggtgactgagacaccgcaaagtgaggtgtaccagtctgggccagactattttttccagaccagtagacaaggcctgcagaccgtaaacctgagccaggctttcaaaaacttgcaggggctgtggggggtgcgggctcccacaggcgaccgcgcgaccgtgtctagcttgctgacgcccaactcgcgcctgttgctgctgctaatagcgcccttcacggacagtggcagcgtgtcccgggacacatacctaggtcacttgctgacactgtaccgcgaggccataggtcaggcgcatgtggacgagcatactttccaggagattacaagtgtcagccgcgcgctggggcaggaggacacgggcagcctggaggcaaccctaaactacctgctgaccaaccggcggcagaagatcccctcgttgcacagtttaaacagcgaggaggagcgcattttgcgctacgtgcagcagagcgtgagccttaacctgatgcgcgacggggtaacgcccagcgtggcgctggacatgaccgcgcgcaacatggaaccgggcatgtatgcctcaaaccggccgtttatcaaccgcctaatggactacttgcatcgcgcggccgccgtgaaccccgagtatttcaccaatgccatcttgaacccgcactggctaccgccccctggtttctacaccgggggattcgaggtgcccgagggtaacgatggattcctctgggacgacatagacgacagcgtgttttccccgcaaccgcagaccctgctagagttgcaacagcgcgagcaggcagaggcggcgctgcgaaaggaaagcttccgcaggccaagcagcttgtccgatctaggcgctgcggccccgcggtcagatgctagtagcccatttccaagcttgatagggtctcttaccagcactcgcaccacccgcccgcgcctgctgggcgaggaggagtacctaaacaactcgctgctgcagccgcagcgcgaaaaaaacctgcctccggcatttcccaacaacgggatagagagcctagtggacaagatgagtagatggaagacgtacgcgcaggagcacagggacgtgccaggcccgcgcccgcccacccgtcgtcaaaggcacgaccgtcagcggggtctggtgtgggaggacgatgactcggcagacgacagcagcgtcctggatttgggagggagtggcaacccgtttgcgcaccttcgccccaggctggggagaatgttttaaaaaaaaaaaagcatgatgcaaaataaaaaactcaccaaggccatggcaccgagcgttggttttcttgtattccccttagtatgcggcgcgcggcgatgtatgaggaaggtcctcctccctcctacgagagtgtggtgagcgcggcgccagtggcggcggcgctgggttctcccttcgatgctcccctggacccgccgtttgtgcctccgcggtacctgcggcctaccggggggagaaacagcatccgttactctgagttggcacccctattcgacaccacccgtgtgtacctggtggacaacaagtcaacggatgtggcatccctgaactaccagaacgaccacagcaactttctgaccacggtcattcaaaacaatgactacagcccgggggaggcaagcacacagaccatcaatcttgacgaccggtcgcactggggcggcgacctgaaaaccatcctgcataccaacatgccaaatgtgaacgagttcatgtttaccaataagtttaaggcgcgggtgatggtgtcgcgcttgcctactaaggacaatcaggtggagctgaaatacgagtgggtggagttcacgctgcccgagggcaactactccgagaccatgaccatagaccttatgaacaacgcgatcgtggagcactacttgaaagtgggcagacagaacggggttctggaaagcgacatcggggtaaagtttgacacccgcaacttcagactggggtttgaccccgtcactggtcttgtcatgcctggggtatatacaaacgaagccttccatccagacatcattttgctgccaggatgcggggtggacttcacccacagccgcctgagcaacttgttgggcatccgcaagcggcaacccttccaggagggctttaggatcacctacgatgatctggagggtggtaacattcccgcactgttggatgtggacgcctaccaggcgagcttgaaagatgacaccgaacagggcgggggtggcgcaggcggcagcaacagcagtggcagcggcgcggaagagaactccaacgcggcagccgcggcaatgcagccggtggaggacatgaacgatcatgccattcgcggcgacacctttgccacacgggctgaggagaagcgcgctgaggccgaagcagcggccgaagctgccgcccccgctgcgcaacccgaggtcgagaagcctcagaagaaaccggtgatcaaacccctgacagaggacagcaagaaacgcagttacaacctaataagcaatgacagcaccttcacccagtaccgcagctggtaccttgcatacaactacggcgaccctcagaccggaatccgctcatggaccctgctttgcactcctgacgtaacctgcggctcggagcaggtctactggtcgttgccagacatgatgcaagaccccgtgaccttccgctccacgcgccagatcagcaactttccggtggtgggcgccgagctgttgcccgtgcactccaagagcttctacaacgaccaggccgtctactcccaactcatccgccagtttacctctctgacccacgtgttcaatcgctttcccgagaaccagattttggcgcgcccgccagcccccaccatcaccaccgtcagtgaaaacgttcctgctctcacagatcacgggacgctaccgctgcgcaacagcatcggaggagtccagcgagtgaccattactgacgccagacgccgcacctgcccctacgtttacaaggccctgggcatagtctcgccgcgcgtcctatcgagccgcactttttgagcaagcatgtccatccttatatcgcccagcaataacacaggctggggcctgcgcttcccaagcaagatgtttggcggggccaagaagcgctccgaccaacacccagtgcgcgtgcgcgggcactaccgcgcgccctggggcgcgcacaaacgcggccgcactgggcgcaccaccgtcgatgacgccatcgacgcggtggtggaggaggcgcgcaactacacgcccacgccgccaccagtgtccacagtggacgcggccattcagaccgtggtgcgcggagcccggcgctatgctaaaatgaagagacggcggaggcgcgtagcacgtcgccaccgccgccgacccggcactgccgcccaacgcgcggcggcggccctgcttaaccgcgcacgtcgcaccggccgacgggcggccatgcgggccgctcgaaggctggccgcgggtattgtcactgtgccccccaggtccaggcgacgagcggccgccgcagcagccgcggccattagtgctatgactcagggtcgcaggggcaacgtgtattgggtgcgcgactcggttagcggcctgcgcgtgcccgtgcgcacccgccccccgcgcaactagattgcaagaaaaaactacttagactcgtactgttgtatgtatccagcggcggcggcgcgcaacgaagctatgtccaagcgcaaaatcaaagaagagatgctccaggtcatcgcgccggagatctatggccccccgaagaaggaagagcaggattacaagccccgaaagctaaagcgggtcaaaaagaaaaagaaagatgatgatgatgaacttgacgacgaggtggaactgctgcacgctaccgcgcccaggcgacgggtacagtggaaaggtcgacgcgtaaaacgtgttttgcgacccggcaccaccgtagtctttacgcccggtgagcgctccacccgcacctacaagcgcgtgtatgatgaggtgtacggcgacgaggacctgcttgagcaggccaacgagcgcctcggggagtttgcctacggaaagcggcataaggacatgctggcgttgccgctggacgagggcaacccaacacctagcctaaagcccgtaacactgcagcaggtgctgcccgcgcttgcaccgtccgaagaaaagcgcggcctaaagcgcgagtctggtgacttggcacccaccgtgcagctgatggtacccaagcgccagcgactggaagatgtcttggaaaaaatgaccgtggaacctgggctggagcccgaggtccgcgtgcggccaatcaagcaggtggcgccgggactgggcgtgcagaccgtggacgttcagatacccactaccagtagcaccagtattgccaccgccacagagggcatggagacacaaacgtccccggttgcctcagcggtggcggatgccgcggtgcaggcggtcgctgcggccgcgtccaagacctctacggaggtgcaaacggacccgtggatgtttcgcgtttcagccccccggcgcccgcgccgttcgaggaagtacggcgccgccagcgcgctactgcccgaatatgccctacatccttccattgcgcctacccccggctatcgtggctacacctaccgccccagaagacgagcaactacccgacgccgaaccaccactggaacccgccgccgccgtcgccgtcgccagcccgtgctggccccgatttccgtgcgcagggtggctcgcgaaggaggcaggaccctggtgctgccaacagcgcgctaccaccccagcatcgtttaaaagccggtctttgtggttcttgcagatatggccctcacctgccgcctccgtttcccggtgccgggattccgaggaagaatgcaccgtaggaggggcatggccggccacggcctgacgggcggcatgcgtcgtgcgcaccaccggcggcggcgcgcgtcgcaccgtcgcatgcgcggcggtatcctgcccctccttattccactgatcgccgcggcgattggcgccgtgcccggaattgcatccgtggccttgcaggcgcagagacactgattaaaaacaagttgcatgtggaaaaatcaaaataaaaagtctggactctcacgctcgcttggtcctgtaactattttgtagaatggaagacatcaactttgcgtctctggccccgcgacacggctcgcgcccgttcatgggaaactggcaagatatcggcaccagcaatatgagcggtggcgccttcagctggggctcgctgtggagcggcattaaaaatttcggttccaccgttaagaactatggcagcaaggcctggaacagcagcacaggccagatgctgagggataagttgaaagagcaaaatttccaacaaaaggtggtagatggcctggcctctggcattagcggggtggtggacctggccaaccaggcagtgcaaaataagattaacagtaagcttgatccccgccctcccgtagaggagcctccaccggccgtggagacagtgtctccagaggggcgtggcgaaaagcgtccgcgccccgacagggaagaaactctggtgacgcaaatagacgagcctccctcgtacgaggaggcactaaagcaaggcctgcccaccacccgtcccatcgcgcccatggctaccggagtgctgggccagcacacacccgtaacgctggacctgcctccccccgccgacacccagcagaaacctgtgctgccaggcccgaccgccgttgttgtaacccgtcctagccgcgcgtccctgcgccgcgccgccagcggtccgcgatcgttgcggcccgtagccagtggcaactggcaaagcacactgaacagcatcgtgggtctgggggtgcaatccctgaagcgccgacgatgcttctgatagctaacgtgtcgtatgtgtgtcatgtatgcgtccatgtcgccgccagaggagctgctgagccgccgcgcgcccgctttccaagatggctaccccttcgatgatgccgcagtggtcttacatgcacatctcgggccaggacgcctcggagtacctgagccccgggctggtgcagtttgcccgcgccaccgagacgtacttcagcctgaataacaagtttagaaaccccacggtggcgcctacgcacgacgtgaccacagaccggtcccagcgtttgacgctgcggttcatccctgtggaccgtgaggatactgcgtactcgtacaaggcgcggttcaccctagctgtgggtgataaccgtgtgctggacatggcttccacgtactttgacatccgcggcgtgctggacaggggccctacttttaagccctactctggcactgcctacaacgccctggctcccaagggtgccccaaatccttgcgaatgggaagagaaaaagaatggaggaggaagcgatgctaatcaaatgcaaactcacgtatttgggcaggcgccttattctggtataaatattacaaaggagggtattcaaataggtattgatgcaaccaaagaggaagataatggaaaggaaatatatgccgataaaacatttcaacctgaacctcaaataggagaatctcagtggcaggatagtgataattactatggagggagagtccttaaaaagactaccccaatgaaaccatgttacggttcatatgcaaaacccacaaatgaaaatggagggcaagctaaattcaaaacacctgaaaaagaaggtgaagaacccaaagaaagtcaagtggaaatgcaatttttcgatattcccagtactggcacaggtggtaatggaacaaatgttaatttcaaacctaaagtggtattgtacagtgaagatgtagatatagaaaccccagacactcatatttcttacatgcccggcaaggaagatgcaagttcacgagaactaatgggccaacaatctatgcccaacaggcctaattacattgcttttagggacaattttattggtctaatgtattacaacagcacgggtaatatgggtgttctggcgggccaagcatcgcagttgaatgctgttgtagatttgcaagacagaaacacagagctttcataccagcttttgcttgattccattggtgatagaaccaggtacttttctatgtggaatcaggctgttgacagctatgatccagatgttagaattattgaaaatcatggaactgaagatgaacttccaaattactgctttccactggatggcgctggaactaacgcagtgtaccaaggtgtaaaagttaaaactactaacaatacagaatgggaaaaagacactgcagtatctgaacacaatcagataagagttggaaataattttgccatggaaatcaatctaaatgccaacctgtggagaaatttcctgtactccaacatagcgctgtatttgcccgacaagctaaagtacagtccttccaacgtaaaaatttctgataacccaaacacctacgactacatgaacaagcgagtggtggctcccgggttagtggactgctacattaaccttggagcacgctggtcccttgactatatggacaacgtcaacccatttaaccaccaccgcaatgctggcctgcgctaccgctcaatgttgctgggcaatggtcgctatgtgcccttccacatccaggtgcctcagaagttctttgccattaaaaacctccttctcctgccgggctcatacacctacgagtggaacttcaggaaggatgttaacatggttctgcagagctccctaggaaatgacctaagggttgacggagccagcattaagtttgatagcatttgcctttacgccaccttcttccccatggcccacaacaccgcctccacgcttgaggccatgcttagaaacgacaccaacgaccagtcctttaacgactatctctccgccgccaacatgctctaccctatacccgccaacgctaccaacgtgcccatatccatcccctcccgcaactgggcggctttccgcggctgggccttcacgcgccttaagactaaggaaaccccatcactgggctcgggctacgacccttattacacctactctggctctataccctacctagatggaaccttttacctcaaccacacctttaagaaggtggccattacctttgactcttctgtcagctggcctggcaatgaccgcctgcttacccccaacgagtttgaaattaagcgctcagttgacggggagggttacaacgttgcccagtgtaacatgaccaaagactggttcctggtacaaatgctagctaactacaacattggctaccagggcttctatatcccagagagctacaaggaccgcatgtactccttctttagaaacttccagcccatgagccgtcaggtggtggatgatactaaatacaaggactaccaacaggtgggcatcctacaccaacacaacaactctggatttgttggctaccttgcccccaccatgcgcgaaggacaggcctaccctgctaacttcccctatccgcttataggcaagaccgcagttgacagcattacccagaaaaagtttctttgcgatcgcaccctttggcgcatcccattctccagtaactttatgtccatgggcgcactcacagacctgggccaaaaccttctctacgccaactccgcccacgcgctagacatgacttttgaggtggatcccatggacgagcccacccttctttatgttttgtttgaagtctttgacgtggtccgtgtgcaccggccgcaccgcggcgtcatcgaaaccgtgtacctgcgcacgcccttctcggccggcaacgccacaacataaagaagcaagcaacatcaacaacagctgccgccatgggctccagtgagcaggaactgaaagccattgtcaaagatcttggttgtgggccatattttttgggcacctatgacaagcgctttccaggctttgtttctccacacaagctcgcctgcgccatagtcaatacggccggtcgcgagactgggggcgtacactggatggcctttgcctggaacccgcactcaaaaacatgctacctctttgagccctttggcttttctgaccagcgactcaagcaggtttaccagtttgagtacgagtcactcctgcgccgtagcgccattgcttcttcccccgaccgctgtataacgctggaaaagtccacccaaagcgtacaggggcccaactcggccgcctgtggactattctgctgcatgtttctccacgcctttgccaactggccccaaactcccatggatcacaaccccaccatgaaccttattaccggggtacccaactccatgctcaacagtccccaggtacagcccaccctgcgtcgcaaccaggaacagctctacagcttcctggagcgccactcgccctacttccgcagccacagtgcgcagattaggagcgccacttctttttgtcacttgaaaaacatgtaaaaataatgtactagagacactttcaataaaggcaaatgcttttatttgtacactctcgggtgattatttacccccacccttgccgtctgcgccgtttaaaaatcaaaggggttctgccgcgcatcgctatgcgccactggcagggacacgttgcgatactggtgtttagtgctccacttaaactcaggcacaaccatccgcggcagctcggtgaagttttcactccacaggctgcgcaccatcaccaacgcgtttagcaggtcgggcgccgatatcttgaagtcgcagttggggcctccgccctgcgcgcgcgagttgcgatacacagggttgcagcactggaacactatcagcgccgggtggtgcacgctggccagcacgctcttgtcggagatcagatccgcgtccaggtcctccgcgttgctcagggcgaacggagtcaactttggtagctgccttcccaaaaagggcgcgtgcccaggctttgagttgcactcgcaccgtagtggcatcaaaaggtgaccgtgcccggtctgggcgttaggatacagcgcctgcataaaagccttgatctgcttaaaagccacctgagcctttgcgccttcagagaagaacatgccgcaagacttgccggaaaactgattggccggacaggccgcgtcgtgcacgcagcaccttgcgtcggtgttggagatctgcaccacatttcggccccaccggttcttcacgatcttggccttgctagactgctccttcagcgcgcgctgcccgttttcgctcgtcacatccatttcaatcacgtgctccttatttatcataatgcttccgtgtagacacttaagctcgccttcgatctcagcgcagcggtgcagccacaacgcgcagcccgtgggctcgtgatgcttgtaggtcacctctgcaaacgactgcaggtacgcctgcaggaatcgccccatcatcgtcacaaaggtcttgttgctggtgaaggtcagctgcaacccgcggtgctcctcgttcagccaggtcttgcatacggccgccagagcttccacttggtcaggcagtagtttgaagttcgcctttagatcgttatccacgtggtacttgtccatcagcgcgcgcgcagcctccatgcccttctcccacgcagacacgatcggcacactcagcgggttcatcaccgtaatttcactttccgcttcgctgggctcttcctcttcctcttgcgtccgcataccacgcgccactgggtcgtcttcattcagccgccgcactgtgcgcttacctcctttgccatgcttgattagcaccggtgggttgctgaaacccaccatttgtagcgccacatcttctctttcttcctcgctgtccacgattacctctggtgatggcgggcgctcgggcttgggagaagggcgcttctttttcttcttgggcgcaatggccaaatccgccgccgaggtcgatggccgcgggctgggtgtgcgcggcaccagcgcgtcttgtgatgagtcttcctcgtcctcggactcgatacgccgcctcatccgcttttttgggggcgcccggggaggcggcggcgacggggacggggacgacacgtcctccatggttgggggacgtcgcgccgcaccgcgtccgcgctcgggggtggtttcgcgctgctcctcttcccgactggccatttccttctcctataggcagaaaaagatcatggagtcagtcgagaagaaggacagcctaaccgccccctctgagttcgccaccaccgcctccaccgatgccgccaacgcgcctaccaccttccccgtcgaggcacccccgcttgaggaggaggaagtgattatcgagcaggacccaggttttgtaagcgaagacgacgaggaccgctcagtaccaacagaggataaaaagcaagaccaggacaacgcagaggcaaacgaggaacaagtcgggcggggggacgaaaggcatggcgactacctagatgtgggagacgacgtgctgttgaagcatctgcagcgccagtgcgccattatctgcgacgcgttgcaagagcgcagcgatgtgcccctcgccatagcggatgtcagccttgcctacgaacgccacctattctcaccgcgcgtaccccccaaacgccaagaaaacggcacatgcgagcccaacccgcgcctcaacttctaccccgtatttgccgtgccagaggtgcttgccacctatcacatctttttccaaaactgcaagatacccctatcctgccgtgccaaccgcagccgagcggacaagcagctggccttgcggcagggcgctgtcatacctgatatcgcctcgctcaacgaagtgccaaaaatctttgagggtcttggacgcgacgagaagcgcgcggcaaacgctctgcaacaggaaaacagcgaaaatgaaagtcactctggagtgttggtggaactcgagggtgacaacgcgcgcctagccgtactaaaacgcagcatcgaggtcacccactttgcctacccggcacttaacctaccccccaaggtcatgagcacagtcatgagtgagctgatcgtgcgccgtgcgcagcccctggagagggatgcaaatttgcaagaacaaacagaggagggcctacccgcagttggcgacgagcagctagcgcgctggcttcaaacgcgcgagcctgccgacttggaggagcgacgcaaactaatgatggccgcagtgctcgttaccgtggagcttgagtgcatgcagcggttctttgctgacccggagatgcagcgcaagctagaggaaacattgcactacacctttcgacagggctacgtacgccaggcctgcaagatctccaacgtggagctctgcaacctggtctcctaccttggaattttgcacgaaaaccgccttgggcaaaacgtgcttcattccacgctcaagggcgaggcgcgccgcgactacgtccgcgactgcgtttacttatttctatgctacacctggcagacggccatgggcgtttggcagcagtgcttggaggagtgcaacctcaaggagctgcagaaactgctaaagcaaaacttgaaggacctatggacggccttcaacgagcgctccgtggccgcgcacctggcggacatcattttccccgaacgcctgcttaaaaccctgcaacagggtctgccagacttcaccagtcaaagcatgttgcagaactttaggaactttatcctagagcgctcaggaatcttgcccgccacctgctgtgcacttcctagcgactttgtgcccattaagtaccgcgaatgccctccgccgctttggggccactgctaccttctgcagctagccaactaccttgcctaccactctgacataatggaagacgtgagcggtgacggtctactggagtgtcactgtcgctgcaacctatgcaccccgcaccgctccctggtttgcaattcgcagctgcttaacgaaagtcaaattatcggtacctttgagctgcagggtccctcgcctgacgaaaagtccgcggctccggggttgaaactcactccggggctgtggacgtcggcttaccttcgcaaatttgtacctgaggactaccacgcccacgagattaggttctacgaagaccaatcccgcccgccaaatgcggagcttaccgcctgcgtcattacccagggccacattcttggccaattgcaagccatcaacaaagcccgccaagagtttctgctacgaaagggacggggggtttacttggacccccagtccggcgaggagctcaacccaatccccccgccgccgcagccctatcagcagcagccgcgggcccttgcttcccaggatggcacccaaaaagaagctgcagctgccgccgccacccacggacgaggaggaatactgggacagtcaggcagaggaggttttggacgaggaggaggaggacatgatggaagactgggagagcctagacgaggaagcttccgaggtcgaagaggtgtcagacgaaacaccgtcaccctcggtcgcattcccctcgccggcgccccagaaatcggcaaccggttccagcatggctacaacctccgctcctcaggcgccgccggcactgcccgttcgccgacccaaccgtagatgggacaccactggaaccagggccggtaagtccaagcagccgccgccgttagcccaagagcaacaacagcgccaaggctaccgctcatggcgcgggcacaagaacgccatagttgcttgcttgcaagactgtgggggcaacatctccttcgcccgccgctttcttctctaccatcacggcgtggccttcccccgtaacatcctgcattactaccgtcatctctacagcccatactgcaccggcggcagcggcagcggcagcaacagcagcggccacacagaagcaaaggcgaccggatagcaagactctgacaaagcccaagaaatccacagcggcggcagcagcaggaggaggagcgctgcgtctggcgcccaacgaacccgtatcgacccgcgagcttagaaacaggatttttcccactctgtatgctatatttcaacagagcaggggccaagaacaagagctgaaaataaaaaacaggtctctgcgatccctcacccgcagctgcctgtatcacaaaagcgaagatcagcttcggcgcacgctggaagacgcggaggctctcttcagtaaatactgcgcgctgactcttaaggactagtttcgcgccctttctcaaatttaagcgcgaaaactacgtcatctccagcggccacacccggcgccagcacctgtcgtcagcgccattatgagcaaggaaattcccacgccctacatgtggagttaccagccacaaatgggacttgcggctggagctgcccaagactactcaacccgaataaactacatgagcgcgggaccccacatgatatcccgggtcaacggaatccgcgcccaccgaaaccgaattctcttggaacaggcggctattaccaccacacctcgtaataaccttaatccccgtagttggcccgctgccctggtgtaccaggaaagtcccgctcccaccactgtggtacttcccagagacgcccaggccgaagttcagatgactaactcaggggcgcagcttgcgggcggctttcgtcacagggtgcggtcgcccgggcagggtataactcacctgacaatcagagggcgaggtattcagctcaacgacgagtcggtgagctcctcgcttggtctccgtccggacgggacatttcagatcggcggcgccggccgtccttcattcacgcctcgtcaggcaatcctaactctgcagacctcgtcctctgagccgcgctctggaggcattggaactctgcaatttattgaggagtttgtgccatcggtctactttaaccccttctcgggacctcccggccactatccggatcaatttattcctaactttgacgcggtaaaggactcggcggacggctacgactgaatgttaagtggagaggcagagcaactgcgcctgaaacacctggtccactgtcgccgccacaagtgctttgcccgcgactccggtgagttttgctactttgaattgcccgaggatcatatcgagggcccggcgcacggcgtccggcttaccgcccagggagagcttgcccgtagcctgattcgggagtttacccagcgccccctgctagttgagcgggacaggggaccctgtgttctcactgtgatttgcaactgtcctaaccttggattacatcaagatctttgttgccatctctgtgctgagtataataaatacagaaattaaaatatactggggctcctatcgccatcctgtaaacgccaccgtcttcacccgcccaagcaaaccaaggcgaaccttacctggtacttttaacatctctccctctgtgatttacaacagtttcaacccagacggagtgagtctacgagagaacctctccgagctcagctactccatcagaaaaaacaccaccctccttacctgccgggaacgtacgagtgcgtcaccggccgctgcaccacacctaccgcctgaccgtaaaccagactttttccggacagacctcaataactctgtttaccagaacaggaggtgagcttagaaaacccttagggtattaggccaaaggcgcagctactgtggggtttatgaacaattcaagcaactctacgggctattctaattcaggtttctctagaatcggggttggggttattctctgtcttgtgattctctttattcttatactaacgcttctctgcctaaggctcgccgcctgctgtgtgcacatttgcatttattgtcagctttttaaacgctggggtcgccacccaagatgattaggtacataatcctaggtttactcacccttgcgtcagcccacggtaccacccaaaaggtggattttaaggagccagcctgtaatgttacattcgcagctgaagctaatgagtgcaccactcttataaaatgcaccacagaacatgaaaagctgcttattcgccacaaaaacaaaattggcaagtatgctgtttatgctatttggcagccaggtgacactacagagtataatgttacagttttccagggtaaaagtcataaaacttttatgtatacttttccattttatgaaatgtgcgacattaccatgtacatgagcaaacagtataagttgtggcccccacaaaattgtgtggaaaacactggcactttctgctgcactgctatgctaattacagtgctcgctttggtctgtaccctactctatattaaatacaaaagcagacgcagctttattgaggaaaagaaaatgccttaatttactaagttacaaagctaatgtcaccactaactgctttactcgctgcttgcaaaacaaattcaaaaagttagcattataattagaataggatttaaaccccccggtcatttcctgctcaataccattcccctgaacaattgactctatgtgggatatgctccagcgctacaaccttgaagtcaggcttcctggatgtcagcatctgactttggccagcacctgtcccgcggatttgttccagtccaactacagcgacccaccctaacagagatgaccaacacaaccaacgcggccgccgctaccggacttacatctaccacaaatacaccccaagtttctgcctttgtcaataactgggataacttgggcatgtggtggttctccatagcgcttatgtttgtatgccttattattatgtggctcatctgctgcctaaagcgcaaacgcgcccgaccacccatctatagtcccatcattgtgctacacccaaacaatgatggaatccatagattggacggactgaaacacatgttcttttctcttacagtatgattaaatgagacatgattcctcgagtttttatattactgacccttgttgcgcttttttgtgcgtgctccacattggctaagtaatagttaattaaacaagtttgtacaaaaaagcaggcttcgaaggagatagaaccaattctctaaggaaatacttaaccatggctctagagatatactgagtcattagggactttccaatgggttttgcccagtacataaggtcaataggggtgaatcaacaggaaagtcccattggagccaagtacactgagtcaatagggactttccattgggttttgcccagtacaaaaggtcaatagggggtgagtcaatgggtttttcccattattggcacgtacataaggtcaataggggtgagtcattgggtttttccagccatttaattaaaacgccatgtactttcccaccattgacgtcaatgggctattgaaactaatgcaacgtgacctttaaacggtactttcccatagctgattaatgggaaagtaccgttctcgagccaatacacgtcaatgggaagtgaaagggcagccaaaacgtaacaccgccccggttttcccctggaaattccatattggcactcattctattggctgagctgcgttctacgtgggtataagaggcgcgaccagcgtcggtaccgtcgcagtcttcggtctgaccaccgtagaacgcagatcgaattactagtcagggaattcgccaccatgtgtcaccagcagttggtcatctcttggttttccctggtttttctggcatctcccctcgtggccatatgggaactgaagaaagatgtttatgtcgtagaattggattggtatccggatgcccctggagaaatggtggtcctcacctgtgacacccctgaagaagatggtatcacctggaccttggaccagagcagtgaggtcttaggctctggcaaaaccctgaccatccaagtcaaagagtttggagatgctggccagtacacctgtcacaaaggaggcgaggttctaagccattcgctcctgctgcttcacaaaaaggaagatggaatttggtccactgatattttaaaggaccagaaagaacccaaaaataagacctttctaagatgcgaggccaagaattattctggacgtttcacctgctggtggctgacgacaatcagtactgatttgacattcagtgtcaaaagcagcagaggctcttctgacccccaaggggtgacgtgcggagctgctacactctctgcagagagagtcagaggggacaacaaggagtatgagtactcagtggagtgccaggaggacagtgcctgcccagctgctgaggagagtctgcccattgaggtcatggtggatgccgttcacaagctcaagtatgaaaactacaccagcagcttcttcatcagggacatcatcaaacctgacccacccaagaacttgcagctgaagccattaaagaactctcggcaggtggaggtcagctgggagtaccctgacacctggagtactccacattcctacttctccctgacattctgcgttcaggtccagggcaagagcaagagagaaaagaaagatagagtcttcacggacaagacctcagccacggtcatctgccgcaaaaatgccagcattagcgtgcgggcccaggaccgctactatagctcatcttggagcgaatgggcatctgtgccctgcagtgttcctggagtaggggtacctggggtgggcgccagaaacctccccgtggccactccagacccaggaatgttcccatgccttcaccactcccaaaacctgctgagggccgtcagcaacatgctccagaaggccagacaaactctagaattttacccttgcacttctgaagagattgatcatgaagacatcacaaaagataaaaccagcacagtggaggcctgtttaccattggaattaaccaagaatgagagttgcctaaattccagagagacctctttcataactaatgggagttgcctggcctccagaaagacctcttttatgatggccctgtgccttagtagtatttatgaagacttgaagatgtaccaggtggagttcaagaccatgaatgcaaagcttctgatggatcctaagaggcagatctttctagatcaaaacatgctggcagttattgatgagctgatgcaggccctgaatttcaacagtgagactgtgccacaaaaatcctcccttgaagaaccggatttttataaaactaaaatcaagctctgcatacttcttcatgctttcagaatacgggcagtgactattgatagagtgatgagctatctgaatgcttcctaattcgagcaacttgtttattgcagcttataatggttacaaataaagcaatagcatcacaaatttcacaaataaagcatttttttcactgcattctagttgtggtttgtccaaactcatcaatgtatcttatcatgtctggatcgtctagcatcgaagatccaaataaaggatcctttatttggatcttcgatgctagacgatccagacatgataagatacattgatgagtttggacaaaccacaactagaatgcagtgaaaaaaatgctttatttgtgaaatttgtgatgctattgctttatttgtaaccattataagctgcaataaacaagttgctcgaatcagctcatctccaaagagttgatgtactcccgaacccatttcttctctgggttggcacacacttggcggttctttcgggtgacaaagacgactgctgggttggagcacttgccactggtgtagaaatactccttgatgtgggcacggggcagtgggcgggcaatgtaggcaaagcagcagggtgtggtgtccgaggaatatggggaggcagatgcaggagcgcagagggcagtagcaatgaggatgacagcgagggctgccgcggagaccttcatggggccagggttctcttccacgtcgccacatgtcagcaggctgcctctgccctctccagatccctgggatgctcttcgacctcgaaacagcatctgactcctttttcgcttccctgttttagctgctggcgacagttcagccatcacttggatgagttcatgtattgctttgcgttggacattcaagtcagttaccgaataattagtcagcttttcgaagtcatctcgtttctttttgttgctattgaaaaacttgacattcatgtcttccttgatggtctccacactcttttggatgctctggtcatctttaaagtttttaaaaagtttgaagtaaaaggagacaatttggctctgcattatttttctgtcactctcctctttccaattcttcaaaatgcctaagaaaagagttccattatccgctacatctgaatgacctgcattaaaatatttcttaaggttttctgcttcttttacatatgggtcctggcagtaacagccaagagaacccaaaacgatgcagagctgaaaagccaagatataacttgtatatttcatggtggccaaaacagcgtggatggcgtctccaggcgatctgacggttcactaaacgagctctgcttatatagacctcccaccgtacacgcctaccgcccatttgcgtcaatggggcggagttgttacgacattttggaaagtcccgttgattttggtgccaaaacaaactcccattgacgtcaatggggtggagacttggaaatccccgtgagtcaaaccgctatccacgcccattgatgtactgccaaaaccgcatcaccatggtaatagcgatgactaatacgtagatgtactgccaagtaggaaagtcccataaggtcatgtactgggcataatgccagggaattagatatctagacccagctttcttgtacaaagtggttaattaagatcttattccctttaactaataaaaaaaaataataaagcatcacttacttaaaatcagttagcaaatttctgtccagtttattcagcagcacctccttgccctcctcccagctctggtattgcagcttcctcctggctgcaaactttctccacaatctaaatggaatgtcagtttcctcctgttcctgtccatccgcacccactatcttcatgttgttgcagatgaagcgcgcaagaccgtctgaagataccttcaaccccgtgtatccatatgacacggaaaccggtcctccaactgtgccttttcttactcctccctttgtatcccccaatgggtttcaagagagtccccctggagttcttactttaaaatgtttaaccccactaacaaccacaggcggatctctacagctaaaagtgggagggggacttacagtggatgacaccaacggttttttgaaagaaaacataagtgccaccacaccactcgttaagactggtcactctataggtttaccactaggagccggattgggaacgaatgaaaataaactttgtatcaaattaggacaaggacttacattcaattcaaacaacatttgcattgatgacaatattaacaccttatggacaggagtcaaccccaccgaagccaactgtcaaatcatgaactccagtgaatctaatgattgcaaattaattctaacactagttaaaactggagcactagtcactgcatttgtttatgttataggagtatctaacaattttaatatgctaactacacacagaaatataaattttactgcagagctgtttttcgattctaactggtaatttaactaactagactctcatcccctcaaaactccacttaatcataaatcaggacaaaacatggctactggtgccattactaatgctaaaggtttcatgcccagcacgactgcctatcctttcaatgataattctagagaaaaagaaaactacatttacggaacttgttactacacagctagtgatcgcactgcttttcccattgacatatctgtcatgcttaaccgaagagcaataaatgacgagacatcatattgtattcgtataacttggtcctggaacacaggagatgccccagaggtgcaaacctctgctacaaccctagtcacctccccatttaccttttactacatcagagaagacgactgagcccaagaataaagaatcgtttgtgttatgtttcaacgtgtttatttttcaattgcagaaaatttcaagtcatttttcattcagtagtatagccccaccaccacatagcttatacagatcaccgtaccttaatcaaactcacagaaccctagtattcaacctgccacctccctcccaacacacagagtacacagtcctttctccccggctggccttaaaaagcatcatatcatgggtaacagacatattcttaggtgttatattccacacggtttcctgtcgagccaaacgctcatcagtgatattaataaactccccgggcagctcacttaagttcatgtcgctgtccagctgctgagccacaggctgctgtccaacttgcggttgcttaacgggcggcgaaggagaagtccacgcctacatgggggtagagtcataatcgtgcatcaggatagggcggtggtgctgcagcagcgcgcgaataaactgctgccgccgccgctccgtcctgcaggaatacaacatggcagtggtctcctcagcgatgattcgcaccgcccgcagcataaggcgccttgtcctccgggcacagcagcgcaccctgatctcacttaaatcagcacagtaactgcagcacagcaccacaatattgttcaaaatcccacagtgcaaggcgctgtatccaaagctcatggcggggaccacagaacccacgtggccatcataccacaagcgcaggtagattaagtggcgacccctcataaacacgctggacataaacattacctcttttggcatgttgtaattcaccacctcccggtaccatataaacctctgattaaacatggcgccatccaccaccatcctaaaccagctggccaaaacctgcccgccggctatacactgcagggaaccgggactggaacaatgacagtggagagcccaggactcgtaaccatggatcatcatgctcgtcatgatatcaatgttggcacaacacaggcacacgtgcatacacttcctcaggattacaagctcctcccgcgttagaaccatatcccagggaacaacccattcctgaatcagcgtaaatcccacactgcagggaagacctcgcacgtaactcacgttgtgcattgtcaaagtgttacattcgggcagcagcggatgatcctccagtatggtagcgcgggtttctgtctcaaaaggaggtagacgatccctactgtacggagtgcgccgagacaaccgagatcgtgttggtcgtagtgtcatgccaaatggaacgccggacgtagtcatatttcctgaagcaaaaccaggtgcgggcgtgacaaacagatctgcgtctccggtctcgccgcttagatcgctctgtgtagtagttgtagtatatccactctctcaaagcatccaggcgccccctggcttcgggttctatgtaaactccttcatgcgccgctgccctgataacatccaccaccgcagaataagccacacccagccaacctacacattcgttctgcgagtcacacacgggaggagcgggaagagctggaagaaccatgtttttttttttattccaaaagattatccaaaacctcaaaatgaagatctattaagtgaacgcgctcccctccggtggcgtggtcaaactctacagccaaagaacagataatggcatttgtaagatgttgcacaatggcttccaaaaggcaaacggccctcacgtccaagtggacgtaaaggctaaacccttcagggtgaatctcctctataaacattccagcaccttcaaccatgcccaaataattctcatctcgccaccttctcaatatatctctaagcaaatcccgaatattaagtccggccattgtaaaaatctgctccagagcgccctccaccttcagcctcaagcagcgaatcatgattgcaaaaattcaggttcctcacagacctgtataagattcaaaagcggaacattaacaaaaataccgcgatcccgtaggtcccttcgcagggccagctgaacataatcgtgcaggtctgcacggaccagcgcggccacttccccgccaggaaccttgacaaaagaacccacactgattatgacacgcatactcggagctatgctaaccagcgtagccccgatgtaagctttgttgcatgggcggcgatataaaatgcaaggtgctgctcaaaaaatcaggcaaagcctcgcgcaaaaaagaaagcacatcgtagtcatgctcatgcagataaaggcaggtaagctccggaaccaccacagaaaaagacaccatttttctctcaaacatgtctgcgggtttctgcataaacacaaaataaaataacaaaaaaacatttaaacattagaagcctgtcttacaacaggaaaaacaacccttataagcataagacggactacggccatgccggcgtgaccgtaaaaaaactggtcaccgtgattaaaaagcaccaccgacagctcctcggtcatgtccggagtcataatgtaagactcggtaaacacatcaggttgattcatcggtcagtgctaaaaagcgaccgaaatagcccgggggaatacatacccgcaggcgtagagacaacattacagcccccataggaggtataacaaaattaataggagagaaaaacacataaacacctgaaaaaccctcctgcctaggcaaaatagcaccctcccgctccagaacaacatacagcgcttcacagcggcagcctaacagtcagccttaccagtaaaaaagaaaacctattaaaaaaacaccactcgacacggcaccagctcaatcagtcacagtgtaaaaaagggccaagtgcagagcgagtatatataggactaaaaaatgacgtaacggttaaagtccacaaaaaacacccagaaaaccgcacgcgaacctacgcccagaaacgaaagccaaaaaacccacaacttcctcaaatcgtcacttccgttttcccacgttacgtaacttcccattttaagaaaactacaattcccaacacatacaagttactccgccctaaaacctacgtcacccgccccgttcccacgccccgcgccacgtcacaaactccaccccctcattatcatattggcttcaatccaaaataaggtatattattgatgat